European Patent Specification EP 3 365 364 B1, published April 10, 2024. Title: ANTIBODY/T-CELL RECEPTOR CHIMERIC CONSTRUCTS AND USES THEREOF. Applicant: Eureka Therapeutics, Inc. Application Not Yet Assigned. The sequence listing filed with the application follows.

SEQUENCE LISTING (82 sequences)

SEQ ID NO: 1 - protein, 20 aa, Homo sapiens
  TCRalpha transmembrane domain
ILLLKVAGFNLLMTLRLWSS

SEQ ID NO: 2 - protein, 23 aa, Homo sapiens
  TCRbeta transmembrane domain
TILYEILLGKATLYAVLVSALVL

SEQ ID NO: 3 - protein, 20 aa, Homo sapiens
  TCRdelta transmembrane domain
MLFAKTVAVNFLLTAKLFFL

SEQ ID NO: 4 - protein, 23 aa, Homo sapiens
  TCRgamma transmembrane domain
YYMYLLLLLKSVVYFAIITCCLL

SEQ ID NO: 5 - protein, 30 aa, Homo sapiens
  TCRalpha connecting peptide
ESSCDVKLVEKSFETDTNLNFQNLSVIGFR

SEQ ID NO: 6 - protein, 17 aa, Homo sapiens
  TCRbeta connecting peptide
ADCGFTSVSYQQGVLSA

SEQ ID NO: 7 - protein, 41 aa, Homo sapiens
  TCRdelta connecting peptide
DHVKPKETENTKQPSKSCHKPKAIVHTEKVNMMSLTVLGLR

SEQ ID NO: 8 - protein, 24 aa, Homo sapiens
  TCRgamma connecting peptide
MDPKDNCSKDANDTLLLQLTNTSA

SEQ ID NO: 9 - protein, 40 aa, Homo sapiens
  TCRalpha connecting peptide MD
IPEDTFFPSPESSCDVKLVEKSFETDTNLNFQNLSVIGFR

SEQ ID NO: 10 - protein, 19 aa, Homo sapiens
  TCRbeta connecting peptide MD
GRADCGFTSVSYQQGVLSA

SEQ ID NO: 11 - protein, 48 aa, Homo sapiens
  TCRdelta connecting peptide MD
EVKTDSTDHVKPKETENTKQPSKSCHKPKAIVHTEKVNMMSLTVLGLR

SEQ ID NO: 12 - protein, 32 aa, Homo sapiens
  TCRgamma connecting peptide MD
PIKTDVITMDPKDNCSKDANDTLLLQLTNTSA

SEQ ID NO: 13 - protein, 9 aa, Homo sapiens
  TCRbeta intracellular domain
MAMVKRKDF

SEQ ID NO: 14 - protein, 12 aa, Homo sapiens
  TCRgamma intracellular domain
RRTAFCCNGEKS

SEQ ID NO: 15 - protein, 50 aa, Homo sapiens
  TCRD alpha
ESSCDVKLVEKSFETDTNLNFQNLSVIGFRILLLKVAGFNLLMTLRLWSS

SEQ ID NO: 16 - protein, 49 aa, Homo sapiens
  TCRD beta
ADCGFTSVSYQQGVLSATILYEILLGKATLYAVLVSALVLMAMVKRKDF

SEQ ID NO: 17 - protein, 60 aa, Homo sapiens
  TCRD alpha MD
IPEDTFFPSPESSCDVKLVEKSFETDTNLNFQNLSVIGFRILLLKVAGFNLLMTLRLWSS

SEQ ID NO: 18 - protein, 51 aa, Homo sapiens
  TCRD beta MD
GRADCGFTSVSYQQGVLSATILYEILLGKATLYAVLVSALVLMAMVKRKDF

SEQ ID NO: 19 - protein, 61 aa, Homo sapiens
  TCRD delta
DHVKPKETENTKQPSKSCHKPKAIVHTEKVNMMSLTVLGLRMLFAKTVAVNFLLTAKLFFL

SEQ ID NO: 20 - protein, 59 aa, Homo sapiens
  TCRD gamma
MDPKDNCSKDANDTLLLQLTNTSAYYMYLLLLLKSVVYFAIITCCLLRRTAFCCNGEKS

SEQ ID NO: 21 - protein, 68 aa, Homo sapiens
  TCRD delta MD
EVKTDSTDHVKPKETENTKQPSKSCHKPKAIVHTEKVNMMSLTVLGLRMLFAKTVAVNFLLTAKLFFL

SEQ ID NO: 22 - protein, 67 aa, Homo sapiens
  TCRD gamma MD
PIKTDVITMDPKDNCSKDANDTLLLQLTNTSAYYMYLLLLLKSVVYFAIITCCLLRRTAFCCNGEKS

SEQ ID NO: 23 - protein, 270 aa, Artificial Sequence
  anti-AFP158/HLA-A*02:01-abTCR-3 alpha
EVQLVQSGAEVKKPGESLTISCKASGYSFPNYWITWVRQMSGGGLEWMGRIDPGDSYTTYNPSFQGHVTISIDKSTNTAYLHWNSLKASDTAMYYCARYYVSLVDIWGQGTLVTVSSASTKGPSVFPLAPSSKSTSGGTAALGCLVKDYFPEPVTVSWNSGALTSGVHTFPAVLQSSGLYSLSSVVTVPSSSLGTQTYICNVNHKPSNTKVDKRVEPKSCESSCDVKLVEKSFETDTNLNFQNLSVIGFRILLLKVAGFNLLMTLRLWSS

SEQ ID NO: 24 - protein, 265 aa, Artificial Sequence
  anti-AFP158/HLA-A*02:01-abTCR-3 beta
QSVLTQPASVSGSPGQSITISCTGTSSDVGGYNYVSWYQQHPGKAPKLMIYDVNNRPSEVSNRFSGSKSGNTASLTISGLQAEDEADYYCSSYTTGSRAVFGGGTKLTVLGQPKANPTVTLFPPSSEELQANKATLVCLISDFYPGAVTVAWKADGSPVKAGVETTKPSKQSNNKYAASSYLSLTPEQWKSHRSYSCQVTHEGSTVEKTVAPTECSADCGFTSVSYQQGVLSATILYEILLGKATLYAVLVSALVLMAMVKRKDF

SEQ ID NO: 25 - protein, 266 aa, Artificial Sequence
  anti-AFP158/HLA-A*02:01-abTCR-4 alpha
QSVLTQPASVSGSPGQSITISCTGTSSDVGGYNYVSWYQQHPGKAPKLMIYDVNNRPSEVSNRFSGSKSGNTASLTISGLQAEDEADYYCSSYTTGSRAVFGGGTKLTVLGQPKANPTVTLFPPSSEELQANKATLVCLISDFYPGAVTVAWKADGSPVKAGVETTKPSKQSNNKYAASSYLSLTPEQWKSHRSYSCQVTHEGSTVEKTVAPTECSESSCDVKLVEKSFETDTNLNFQNLSVIGFRILLLKVAGFNLLMTLRLWSS

SEQ ID NO: 26 - protein, 269 aa, Artificial Sequence
  anti-AFP158/HLA-A*02:01-abTCR-4 beta
EVQLVQSGAEVKKPGESLTISCKASGYSFPNYWITWVRQMSGGGLEWMGRIDPGDSYTTYNPSFQGHVTISIDKSTNTAYLHWNSLKASDTAMYYCARYYVSLVDIWGQGTLVTVSSASTKGPSVFPLAPSSKSTSGGTAALGCLVKDYFPEPVTVSWNSGALTSGVHTFPAVLQSSGLYSLSSVVTVPSSSLGTQTYICNVNHKPSNTKVDKRVEPKSCADCGFTSVSYQQGVLSATILYEILLGKATLYAVLVSALVLMAMVKRKDF

SEQ ID NO: 27 - protein, 276 aa, Artificial Sequence
  anti-AFP158/HLA-A*02:01-abTCR-4MD alpha
QSVLTQPASVSGSPGQSITISCTGTSSDVGGYNYVSWYQQHPGKAPKLMIYDVNNRPSEVSNRFSGSKSGNTASLTISGLQAEDEADYYCSSYTTGSRAVFGGGTKLTVLGQPKANPTVTLFPPSSEELQANKATLVCLISDFYPGAVTVAWKADGSPVKAGVETTKPSKQSNNKYAASSYLSLTPEQWKSHRSYSCQVTHEGSTVEKTVAPTECSIPEDTFFPSPESSCDVKLVEKSFETDTNLNFQNLSVIGFRILLLKVAGFNLLMTLRLWSS

SEQ ID NO: 28 - protein, 271 aa, Artificial Sequence
  anti-AFP158/HLA-A*02:01-abTCR-4MD beta
EVQLVQSGAEVKKPGESLTISCKASGYSFPNYWITWVRQMSGGGLEWMGRIDPGDSYTTYNPSFQGHVTISIDKSTNTAYLHWNSLKASDTAMYYCARYYVSLVDIWGQGTLVTVSSASTKGPSVFPLAPSSKSTSGGTAALGCLVKDYFPEPVTVSWNSGALTSGVHTFPAVLQSSGLYSLSSVVTVPSSSLGTQTYICNVNHKPSNTKVDKRVEPKSCGRADCGFTSVSYQQGVLSATILYEILLGKATLYAVLVSALVLMAMVKRKDF

SEQ ID NO: 29 - protein, 277 aa, Artificial Sequence
  anti-AFP158/HLA-A*02:01-abTCR-5 delta
QSVLTQPASVSGSPGQSITISCTGTSSDVGGYNYVSWYQQHPGKAPKLMIYDVNNRPSEVSNRFSGSKSGNTASLTISGLQAEDEADYYCSSYTTGSRAVFGGGTKLTVLGQPKANPTVTLFPPSSEELQANKATLVCLISDFYPGAVTVAWKADGSPVKAGVETTKPSKQSNNKYAASSYLSLTPEQWKSHRSYSCQVTHEGSTVEKTVAPTECSDHVKPKETENTKQPSKSCHKPKAIVHTEKVNMMSLTVLGLRMLFAKTVAVNFLLTAKLFFL

SEQ ID NO: 30 - protein, 279 aa, Artificial Sequence
  anti-AFP158/HLA-A*02:01-abTCR-5 gamma
EVQLVQSGAEVKKPGESLTISCKASGYSFPNYWITWVRQMSGGGLEWMGRIDPGDSYTTYNPSFQGHVTISIDKSTNTAYLHWNSLKASDTAMYYCARYYVSLVDIWGQGTLVTVSSASTKGPSVFPLAPSSKSTSGGTAALGCLVKDYFPEPVTVSWNSGALTSGVHTFPAVLQSSGLYSLSSVVTVPSSSLGTQTYICNVNHKPSNTKVDKRVEPKSCMDPKDNCSKDANDTLLLQLTNTSAYYMYLLLLLKSVVYFAIITCCLLRRTAFCCNGEKS

SEQ ID NO: 31 - protein, 284 aa, Artificial Sequence
  anti-AFP158/HLA-A*02:01-abTCR-5MD delta
QSVLTQPASVSGSPGQSITISCTGTSSDVGGYNYVSWYQQHPGKAPKLMIYDVNNRPSEVSNRFSGSKSGNTASLTISGLQAEDEADYYCSSYTTGSRAVFGGGTKLTVLGQPKANPTVTLFPPSSEELQANKATLVCLISDFYPGAVTVAWKADGSPVKAGVETTKPSKQSNNKYAASSYLSLTPEQWKSHRSYSCQVTHEGSTVEKTVAPTECSEVKTDSTDHVKPKETENTKQPSKSCHKPKAIVHTEKVNMMSLTVLGLRMLFAKTVAVNFLLTAKLFFL

SEQ ID NO: 32 - protein, 287 aa, Artificial Sequence
  anti-AFP158/HLA-A*02:01-abTCR-5MD gamma
EVQLVQSGAEVKKPGESLTISCKASGYSFPNYWITWVRQMSGGGLEWMGRIDPGDSYTTYNPSFQGHVTISIDKSTNTAYLHWNSLKASDTAMYYCARYYVSLVDIWGQGTLVTVSSASTKGPSVFPLAPSSKSTSGGTAALGCLVKDYFPEPVTVSWNSGALTSGVHTFPAVLQSSGLYSLSSVVTVPSSSLGTQTYICNVNHKPSNTKVDKRVEPKSCPIKTDVITMDPKDNCSKDANDTLLLQLTNTSAYYMYLLLLLKSVVYFAIITCCLLRRTAFCCNGEKS

SEQ ID NO: 33 - protein, 281 aa, Artificial Sequence
  anti-AFP158/HLA-A*02:01-abTCR-6 delta
EVQLVQSGAEVKKPGESLTISCKASGYSFPNYWITWVRQMSGGGLEWMGRIDPGDSYTTYNPSFQGHVTISIDKSTNTAYLHWNSLKASDTAMYYCARYYVSLVDIWGQGTLVTVSSASTKGPSVFPLAPSSKSTSGGTAALGCLVKDYFPEPVTVSWNSGALTSGVHTFPAVLQSSGLYSLSSVVTVPSSSLGTQTYICNVNHKPSNTKVDKRVEPKSCDHVKPKETENTKQPSKSCHKPKAIVHTEKVNMMSLTVLGLRMLFAKTVAVNFLLTAKLFFL

SEQ ID NO: 34 - protein, 275 aa, Artificial Sequence
  anti-AFP158/HLA-A*02:01-abTCR-6 gamma
QSVLTQPASVSGSPGQSITISCTGTSSDVGGYNYVSWYQQHPGKAPKLMIYDVNNRPSEVSNRFSGSKSGNTASLTISGLQAEDEADYYCSSYTTGSRAVFGGGTKLTVLGQPKANPTVTLFPPSSEELQANKATLVCLISDFYPGAVTVAWKADGSPVKAGVETTKPSKQSNNKYAASSYLSLTPEQWKSHRSYSCQVTHEGSTVEKTVAPTECSMDPKDNCSKDANDTLLLQLTNTSAYYMYLLLLLKSVVYFAIITCCLLRRTAFCCNGEKS

SEQ ID NO: 35 - protein, 288 aa, Artificial Sequence
  anti-AFP158/HLA-A*02:01-abTCR-6MD delta
EVQLVQSGAEVKKPGESLTISCKASGYSFPNYWITWVRQMSGGGLEWMGRIDPGDSYTTYNPSFQGHVTISIDKSTNTAYLHWNSLKASDTAMYYCARYYVSLVDIWGQGTLVTVSSASTKGPSVFPLAPSSKSTSGGTAALGCLVKDYFPEPVTVSWNSGALTSGVHTFPAVLQSSGLYSLSSVVTVPSSSLGTQTYICNVNHKPSNTKVDKRVEPKSCEVKTDSTDHVKPKETENTKQPSKSCHKPKAIVHTEKVNMMSLTVLGLRMLFAKTVAVNFLLTAKLFFL

SEQ ID NO: 36 - protein, 283 aa, Artificial Sequence
  anti-AFP158/HLA-A*02:01-abTCR-6MD gamma
QSVLTQPASVSGSPGQSITISCTGTSSDVGGYNYVSWYQQHPGKAPKLMIYDVNNRPSEVSNRFSGSKSGNTASLTISGLQAEDEADYYCSSYTTGSRAVFGGGTKLTVLGQPKANPTVTLFPPSSEELQANKATLVCLISDFYPGAVTVAWKADGSPVKAGVETTKPSKQSNNKYAASSYLSLTPEQWKSHRSYSCQVTHEGSTVEKTVAPTECSPIKTDVITMDPKDNCSKDANDTLLLQLTNTSAYYMYLLLLLKSVVYFAIITCCLLRRTAFCCNGEKS

SEQ ID NO: 37 - protein, 471 aa, Artificial Sequence
  anti-AFP158/HLA-A*02:01-scFv CAR
QSVLTQPASVSGSPGQSITISCTGTSSDVGGYNYVSWYQQHPGKAPKLMIYDVNNRPSEVSNRFSGSKSGNTASLTISGLQAEDEADYYCSSYTTGSRAVFGGGTKLTVLGSRGGGGSGGGGSGGGGSLEMAEVQLVQSGAEVKKPGESLTISCKASGYSFPNYWITWVRQMSGGGLEWMGRIDPGDSYTTYNPSFQGHVTISIDKSTNTAYLHWNSLKASDTAMYYCARYYVSLVDIWGQGTLVTVSSAAAIEVMYPPPYLDNEKSNGTIIHVKGKHLCPSPLFPGPSKPFWVLVVVGGVLACYSLLVTVAFIIFWVRSKRSRLLHSDYMNMTPRRPGPTRKHYQPYAPPRDFAAYRSRVKFSRSADAPAYQQGQNQLYNELNLGRREEYDVLDKRRGRDPEMGGKPRRKNPQEGLYNELQKDKMAEAYSEIGMKGERRRGKGHDGLYQGLSTATKDTYDALHMQALPPR

SEQ ID NO: 38 - protein, 117 aa, Artificial Sequence
  IgVH domain of anti-AFP158/HLA-A*02:01 antibody
EVQLVQSGAEVKKPGESLTISCKASGYSFPNYWITWVRQMSGGGLEWMGRIDPGDSYTTYNPSFQGHVTISIDKSTNTAYLHWNSLKASDTAMYYCARYYVSLVDIWGQGTLVTVSS

SEQ ID NO: 39 - protein, 103 aa, Homo sapiens
  IgG1 CH1 domain
ASTKGPSVFPLAPSSKSTSGGTAALGCLVKDYFPEPVTVSWNSGALTSGVHTFPAVLQSSGLYSLSSVVTVPSSSLGTQTYICNVNHKPSNTKVDKRVEPKSC

SEQ ID NO: 40 - protein, 110 aa, Artificial Sequence
  IgVL domain of AFP158/HLA-A*02:01 antibody
QSVLTQPASVSGSPGQSITISCTGTSSDVGGYNYVSWYQQHPGKAPKLMIYDVNNRPSEVSNRFSGSKSGNTASLTISGLQAEDEADYYCSSYTTGSRAVFGGGTKLTVL

SEQ ID NO: 41 - protein, 106 aa, Homo sapiens
  IgCL domain
GQPKANPTVTLFPPSSEELQANKATLVCLISDFYPGAVTVAWKADGSPVKAGVETTKPSKQSNNKYAASSYLSLTPEQWKSHRSYSCQVTHEGSTVEKTVAPTECS

SEQ ID NO: 42 - protein, 301 aa, Artificial Sequence
  anti-CD19-abTCR-6MD delta
EVQLVQSGAEVKKPGESLKISCKGSGYSFTSYWIGWVRQMPGKGLEWMGIIYPGDSDTRYSPSFQGQVTISADKSISTAYLQWSSLKASDTAMYYCARQVWGWQGGMYPRSNWWYNMDSWGQGTLVTVSSASTKGPSVFPLAPSSKSTSGGTAALGCLVKDYFPEPVTVSWNSGALTSGVHTFPAVLQSSGLYSLSSVVTVPSSSLGTQTYICNVNHKPSNTKVDKRVEPKSCEVKTDSTDHVKPKETENTKQPSKSCHKPKAIVHTEKVNMMSLTVLGLRMLFAKTVAVNFLLTAKLFFL

SEQ ID NO: 43 - protein, 281 aa, Artificial Sequence
  anti-CD19-abTCR-6MD gamma
LPVLTQPPSVSVAPGKTARITCGGNNIGSKSVHWYQQKPGQAPVLVVYDDSNRPSGIPERFSGSNSGNTATLTISRVEAGDEADYYCQVWDSSSEYVVFGGGTKLTVLGQPKANPTVTLFPPSSEELQANKATLVCLISDFYPGAVTVAWKADGSPVKAGVETTKPSKQSNNKYAASSYLSLTPEQWKSHRSYSCQVTHEGSTVEKTVAPTECSPIKTDVITMDPKDNCSKDANDTLLLQLTNTSAYYMYLLLLLKSVVYFAIITCCLLRRTAFCCNGEKS

SEQ ID NO: 44 - protein, 482 aa, Artificial Sequence
  anti-CD19-scFv CAR
LPVLTQPPSVSVAPGKTARITCGGNNIGSKSVHWYQQKPGQAPVLVVYDDSNRPSGIPERFSGSNSGNTATLTISRVEAGDEADYYCQVWDSSSEYVVFGGGTKLTVLGSRGGGGSGGGGSGGGGSLEMAEVQLVQSGAEVKKPGESLKISCKGSGYSFTSYWIGWVRQMPGKGLEWMGIIYPGDSDTRYSPSFQGQVTISADKSISTAYLQWSSLKASDTAMYYCARQVWGWQGGMYPRSNWWYNMDSWGQGTLVTVSSAAAIEVMYPPPYLDNEKSNGTIIHVKGKHLCPSPLFPGPSKPFWVLVVVGGVLACYSLLVTVAFIIFWVRSKRSRLLHSDYMNMTPRRPGPTRKHYQPYAPPRDFAAYRSRVKFSRSADAPAYQQGQNQLYNELNLGRREEYDVLDKRRGRDPEMGGKPRRKNPQEGLYNELQKDKMAEAYSEIGMKGERRRGKGHDGLYQGLSTATKDTYDALHMQALPPR

SEQ ID NO: 45 - protein, 130 aa, Artificial Sequence
  IgVH domain of anti-CD19 antibody
EVQLVQSGAEVKKPGESLKISCKGSGYSFTSYWIGWVRQMPGKGLEWMGIIYPGDSDTRYSPSFQGQVTISADKSISTAYLQWSSLKASDTAMYYCARQVWGWQGGMYPRSNWWYNMDSWGQGTLVTVSS

SEQ ID NO: 46 - protein, 108 aa, Artificial Sequence
  IgVL domain of anti-CD19 antibody
LPVLTQPPSVSVAPGKTARITCGGNNIGSKSVHWYQQKPGQAPVLVVYDDSNRPSGIPERFSGSNSGNTATLTISRVEAGDEADYYCQVWDSSSEYVVFGGGTKLTVL

SEQ ID NO: 47 - protein, 107 aa, Homo sapiens
  fragment of CD28
IEVMYPPPYLDNEKSNGTIIHVKGKHLCPSPLFPGPSKPFWVLVVVGGVLACYSLLVTVAFIIFWVRSKRSRLLHSDYMNMTPRRPGPTRKHYQPYAPPRDFAAYRS

SEQ ID NO: 48 - protein, 112 aa, Homo sapiens
  fragment of CD3-zeta
RVKFSRSADAPAYQQGQNQLYNELNLGRREEYDVLDKRRGRDPEMGGKPRRKNPQEGLYNELQKDKMAEAYSEIGMKGERRRGKGHDGLYQGLSTATKDTYDALHMQALPPR

SEQ ID NO: 49 - protein, 20 aa, Homo sapiens
  Signal peptide
METDTLLLWVLLLWVPGSTG

SEQ ID NO: 50 - protein, 9 aa, Artificial Sequence
  HA tag
YPYDVPDYA

SEQ ID NO: 51 - protein, 22 aa, Artificial Sequence
  3x Flag tag
DYKDHDGDYKDHDIDYKDDDDK

SEQ ID NO: 52 - protein, 10 aa, Artificial Sequence
  myc tag
EQKLISEEDL

SEQ ID NO: 53 - protein, 9 aa, Homo sapiens
  AFP158
FMNKFIYEI

SEQ ID NO: 54 - protein, 281 aa, Artificial Sequence
  anti-CD19 clone 5 abTCR-6MD gamma
LPVLTQPPSVSVAPGKTARITCGGNNIGSKSVHWYQQKPGQAPVLVVYDDSDRPSGIPERFSGSNSGNTATLTISRVEAGDEADYYCQVWDSSSDYVVFGGGTKLTVLGQPKANPTVTLFPPSSEELQANKATLVCLISDFYPGAVTVAWKADGSPVKAGVETTKPSKQSNNKYAASSYLSLTPEQWKSHRSYSCQVTHEGSTVEKTVAPTECSPIKTDVITMDPKDNCSKDANDTLLLQLTNTSAYYMYLLLLLKSVVYFAIITCCLLRRTAFCCNGEKS

SEQ ID NO: 55 - protein, 301 aa, Artificial Sequence
  anti-CD19 clone 5-9 abTCR-6MD delta
EVQLVQSGAEVKKPGESLKISCKGSGYSFTSYWIGWVRQMPGKGLEWMGIIYPGDSDTRYSPFFQGQVTISADKSISTAYLQWSSLKASDTAMYYCARQVWGWQGGMYPRSNWWYNMDSWGQGTLVTVSSASTKGPSVFPLAPSSKSTSGGTAALGCLVKDYFPEPVTVSWNSGALTSGVHTFPAVLQSSGLYSLSSVVTVPSSSLGTQTYICNVNHKPSNTKVDKRVEPKSCEVKTDSTDHVKPKETENTKQPSKSCHKPKAIVHTEKVNMMSLTVLGLRMLFAKTVAVNFLLTAKLFFL

SEQ ID NO: 56 - protein, 301 aa, Artificial Sequence
  anti-CD19 clone 5-13 abTCR-6MD delta
EVQLVQSGAEVKKPGESLKISCKGSGYSFTSYWIGWVRQMPGKGLEWMGIIYPGDSDTRYSPSFQGQVTISADKSISTAYLQWSSLKASDTAMYYCARQVWGWQGGMYPRSNWWYNLDSWGQGTLVTVSSASTKGPSVFPLAPSSKSTSGGTAALGCLVKDYFPEPVTVSWNSGALTSGVHTFPAVLQSSGLYSLSSVVTVPSSSLGTQTYICNVNHKPSNTKVDKRVEPKSCEVKTDSTDHVKPKETENTKQPSKSCHKPKAIVHTEKVNMMSLTVLGLRMLFAKTVAVNFLLTAKLFFL

SEQ ID NO: 57 - protein, 108 aa, Artificial Sequence
  IgVL domain of anti-CD19 antibody clone 5
LPVLTQPPSVSVAPGKTARITCGGNNIGSKSVHWYQQKPGQAPVLVVYDDSDRPSGIPERFSGSNSGNTATLTISRVEAGDEADYYCQVWDSSSDYVVFGGGTKLTVL

SEQ ID NO: 58 - protein, 130 aa, Artificial Sequence
  IgVH domain of anti-CD19 antibody clone 5-9
EVQLVQSGAEVKKPGESLKISCKGSGYSFTSYWIGWVRQMPGKGLEWMGIIYPGDSDTRYSPFFQGQVTISADKSISTAYLQWSSLKASDTAMYYCARQVWGWQGGMYPRSNWWYNMDSWGQGTLVTVSS

SEQ ID NO: 59 - protein, 130 aa, Artificial Sequence
  IgVH domain of anti-CD19 antibody clone 5-13
EVQLVQSGAEVKKPGESLKISCKGSGYSFTSYWIGWVRQMPGKGLEWMGIIYPGDSDTRYSPSFQGQVTISADKSISTAYLQWSSLKASDTAMYYCARQVWGWQGGMYPRSNWWYNLDSWGQGTLVTVSS

SEQ ID NO: 60 - protein, 101 aa, Homo sapiens
  IgG2-0C CH1
ASTKGPSVFPLAPCSRSTSESTAALGCLVKDYFPEPVTVSWNSGALTSGVHTFPAVLQSSGLYSLSSVVTVPSSNFGTQTYTCNVDHKPSNTKVDKTVERK

SEQ ID NO: 61 - protein, 102 aa, Homo sapiens
  IgG2-1C CH1
ASTKGPSVFPLAPCSRSTSESTAALGCLVKDYFPEPVTVSWNSGALTSGVHTFPAVLQSSGLYSLSSVVTVPSSNFGTQTYTCNVDHKPSNTKVDKTVERKC

SEQ ID NO: 62 - protein, 103 aa, Homo sapiens
  IgG2-2C CH1
ASTKGPSVFPLAPCSRSTSESTAALGCLVKDYFPEPVTVSWNSGALTSGVHTFPAVLQSSGLYSLSSVVTVPSSNFGTQTYTCNVDHKPSNTKVDKTVERKCC

SEQ ID NO: 63 - protein, 103 aa, Homo sapiens
  IgG3 CH1
ASTKGPSVFPLAPCSRSTSGGTAALGCLVKDYFPEPVTVSWNSGALTSGVHTFPAVLQSSGLYSLSSVVTVPSSSLGTQTYTCNVNHKPSNTKVDKRVELKTP

SEQ ID NO: 64 - protein, 103 aa, Homo sapiens
  IgG4 CH1
ASTKGPSVFPLAPCSRSTSESTAALGCLVKDYFPEPVTVSWNSGALTSGVHTFPAVLQSSGLYSLSSVVTVPSSSLGTKTYTCNVDHKPSNTKVDKRVESKYG

SEQ ID NO: 65 - protein, 121 aa, Homo sapiens
  IgA1 CH1
ASPTSPKVFPLSLCSTQPDGNVVIACLVQGFFPQEPLSVTWSESGQGVTARNFPPSQDASGDLYTTSSQLTLPATQCLAGKSVTCHVKHYTNPSQDVTVPCPVPSTPPTPSPSTPPTPSPS

SEQ ID NO: 66 - protein, 108 aa, Homo sapiens
  IgA2 CH1
ASPTSPKVFPLSLDSTPQDGNVVVACLVQGFFPQEPLSVTWSESGQNVTARNFPPSQDASGDLYTTSSQLTLPATQCPDGKSVTCHVKHYTNPSQDVTVPCPVPPPPP

SEQ ID NO: 67 - protein, 159 aa, Homo sapiens
  IgD CH1
APTKAPDVFPIISGCRHPKDNSPVVLACLITGYHPTSVTVTWYMGTQSQPQRTFPEIQRRDSYYMTSSQLSTPLQQWRQGEYKCVVQHTASKSKKEIFRWPESPKAQASSVPTAQPQAEGSLAKATTAPATTRNTGRGGEEKKKEKEKEEQEERETKTP

SEQ ID NO: 68 - protein, 103 aa, Homo sapiens
  IgE CH1
ASTQSPSVFPLTRCCKNIPSNATSVTLGCLATGYFPEPVMVTWDTGSLNGTTMTLPATTLTLSGHYATISLLTVSGAWAKQMFTCRVAHTPSSTDWVDNKTFS

SEQ ID NO: 69 - protein, 104 aa, Homo sapiens
  IgM CH1
GSASAPTLFPLVSCENSPSDTSSVAVGCLAQDFLPDSITLSWKYKNNSDISSTRGFPSVLRGGKYAATSQVLLPSKDVMQGTDEHVVCKVQHPNGNKEKNVPLP

SEQ ID NO: 70 - protein, 41 aa, Homo sapiens
  CD28 co-stimulatory fragment
RSKRSRLLHSDYMNMTPRRPGPTRKHYQPYAPPRDFAAYRS

SEQ ID NO: 71 - protein, 42 aa, Homo sapiens
  4-1BB co-stimulatory fragment
KRGRKKLLYIFKQPFMRPVQTTQEEDGCSCRFPEEEEGGCEL

SEQ ID NO: 72 - protein, 117 aa, Artificial Sequence
  IgVH domain of anti-NY-ESO-1/HLA-A*02:01 antibody clone 35
QVQLVQSGAEVKKPGSSVKVSCKASGDTFSSYSISWVRQAPGQGLEWMGRIIPILGIANYAQKYQGRVTLSADKSTSTSYMELNSLRSEDTAVYYCARDWSYSIDYWGQGTLVTVSS

SEQ ID NO: 73 - protein, 111 aa, Artificial Sequence
  IgVL domain of anti-NY-ESO-1/HLA-A*02:01 antibody clone 35
QSVVTQPPSVSAAPGQKVTISCSGSSSNIGNNYVSWYQQLPGTAPKLLIYDNNKRPSGIPDRFSGSKSGTSATLGITGLQTGDEADYYCGTWDSSLSAWVFGGGTKLTVLG

SEQ ID NO: 74 - protein, 21 aa, Artificial Sequence
  scFv linker
SRGGGGSGGGGSGGGGSLEMA

SEQ ID NO: 75 - protein, 284 aa, Artificial Sequence
  anti-CD19-cTCR delta
EVQLVQSGAEVKKPGESLKISCKGSGYSFTSYWIGWVRQMPGKGLEWMGIIYPGDSDTRYSPSFQGQVTISADKSISTAYLQWSSLKASDTAMYYCARQVWGWQGGMYPRSNWWYNLDSWGQGTLVTVSSRSQPHTKPSVFVMKNGTNVACLVKEFYPKDIRINLVSSKKITEFDPAIVISPSGKYNAVKLGKYEDSNSVTCSVQHDNKTVHSTDFEVKTDSTDHVKPKETENTKQPSKSCHKPKAIVHTEKVNMMSLTVLGLRMLFAKTVAVNFLLTAKLFFL

SEQ ID NO: 76 - protein, 282 aa, Artificial Sequence
  anti-CD19-cTCR gamma
LPVLTQPPSVSVAPGKTARITCGGNNIGSKSVHWYQQKPGQAPVLVVYDDSDRPSGIPERFSGSNSGNTATLTISRVEAGDEADYYCQVWDSSSDYVVFGGGTKLTVLGDKQLDADVSPKPTIFLPSIAETKLQKAGTYLCLLEKFFPDVIKIHWQEKKSNTILGSQEGNTMKTNDTYMKFSWLTVPEKSLDKEHRCIVRHENNKNGVDQEIIFPPIKTDVITMDPKDNCSKDANDTLLLQLTNTSAYYMYLLLLLKSVVYFAIITCCLLRRTAFCCNGEKS

SEQ ID NO: 77 - protein, 142 aa, Homo sapiens
  TCRalpha constant domain
PNIQNPDPAVYQLRDSKSSDKSVCLFTDFDSQTNVSQSKDSDVYITDKTVLDMRSMDFKSNSAVAWSNKSDFACANAFNNSIIPEDTFFPSPESSCDVKLVEKSFETDTNLNFQNLSVIGFRILLLKVAGFNLLMTLRLWSS

SEQ ID NO: 78 - protein, 177 aa, Homo sapiens
  TCRbeta constant domain
EDLNKVFPPEVAVFEPSEAEISHTQKATLVCLATGFFPDHVELSWWVNGKEVHSGVSTDPQPLKEQPALNDSRYCLSSRLRVSATFWQNPRNHFRCQVQFYGLSENDEWTQDRAKPVTQIVSAEAWGRADCGFTSVSYQQGVLSATILYEILLGKATLYAVLVSALVLMAMVKRKDF

SEQ ID NO: 79 - protein, 153 aa, Homo sapiens
  TCRdelta constant domain
SQPHTKPSVFVMKNGTNVACLVKEFYPKDIRINLVSSKKITEFDPAIVISPSGKYNAVKLGKYEDSNSVTCSVQHDNKTVHSTDFEVKTDSTDHVKPKETENTKQPSKSCHKPKAIVHTEKVNMMSLTVLGLRMLFAKTVAVNFLLTAKLFFL

SEQ ID NO: 80 - protein, 173 aa, Homo sapiens
  TCRgamma constant domain
DKQLDADVSPKPTIFLPSIAETKLQKAGTYLCLLEKFFPDVIKIHWQEKKSNTILGSQEGNTMKTNDTYMKFSWLTVPEKSLDKEHRCIVRHENNKNGVDQEIIFPPIKTDVITMDPKDNCSKDANDTLLLQLTNTSAYYMYLLLLLKSVVYFAIITCCLLRRTAFCCNGEKS

SEQ ID NO: 81 - protein, 271 aa, Artificial Sequence
  anti-AFP158/HLA-A*02:01 abTCR-7 delta
EVQLVQSGAEVKKPGESLTISCKASGYSFPNYWITWVRQMSGGGLEWMGRIDPGDSYTTYNPSFQGHVTISIDKSTNTAYLHWNSLKASDTAMYYCARYYVSLVDIWGQGTLVTVSSRSQPHTKPSVFVMKNGTNVACLVKEFYPKDIRINLVSSKKITEFDPAIVISPSGKYNAVKLGKYEDSNSVTCSVQHDNKTVHSTDFEVKTDSTDHVKPKETENTKQPSKSCHKPKAIVHTEKVNMMSLTVLGLRMLFAKTVAVNFLLTAKLFFL

SEQ ID NO: 82 - protein, 283 aa, Artificial Sequence
  anti-AFP158/HLA-A*02:01 abTCR-7 gamma
QSVLTQPASVSGSPGQSITISCTGTSSDVGGYNYVSWYQQHPGKAPKLMIYDVNNRPSEVSNRFSGSKSGNTASLTISGLQAEDEADYYCSSYTTGSRAVFGGGTKLTVLDKQLDADVSPKPTIFLPSIAETKLQKAGTYLCLLEKFFPDVIKIHWQEKKSNTILGSQEGNTMKTNDTYMKFSWLTVPEKSLDKEHRCIVRHENNKNGVDQEIIFPPIKTDVITMDPKDNCSKDANDTLLLQLTNTSAYYMYLLLLLKSVVYFAIITCCLLRRTAFCCNGEKS